European Patent Application EP 4 782 544 A1, published July 29, 2026. Title: Microorganism having enhanced activity of aromatic amino acid transporter and uses thereof. Applicant: CJ CheilJedang Corporation. The sequence listing filed with the application follows.

SEQUENCE LISTING (23 sequences)

SEQ ID NO: 1 - protein, 463 aa, synthetic construct
  REGION 1..463: note = aroP protein (NCBI Sequence ID: WP_003863791.1)
MAKSNEGLGTGLRTRHLTMMGLGSAIGAGLFLGTGVGIRAAGPAVLLAYIIAGAIVVLVMQMLGEMAAARPASGSFSRYGEDAFGHWAGFSLGWLYWFMLIMVMGAEMTGAAAIMGAWFGVEPWIPSLVCVVFFAVVNLVAVRGFGEFEYWFAFIKVAVIIAFLIIGIALIFGWLPGSTFVGTSNFIGDHGFMPNGISGVAAGLLAVAFAFGGIEIVTIAAAESDKPREAISLAVRAVIWRISVFYLGSVLVITFLMPYESINGADTAAESPFTQILAMANIPGTVGFMEAIIVLALLSAFNAQIYATSRLVFSMANRQDAPRVFSKLSTSHVPTNAVLLSMFFAFVSVGLQYWNPAGLLDFLLNAVGGCLIVVWAMITLSQLKLRKELQANGEISTVRMWAHPWLGILTLVLLAGLVALMLGDAASRSQVYSVAIVYGFLVLLSFVTVNSPLRGGRTPSDLN

SEQ ID NO: 2 - DNA, 1392 bp, synthetic construct
  misc_feature 1..1392: note = gene coding aroP protein
  source 1..1392: mol_type = other DNA
atggctaaatctaatgaagggctgggaaccggacttcggacccgccacctcacaatgatgggactcggctccgcaattggtgccggactgttcctcggcaccggcgttggtatccgcgcagctggccccgcagtgctcctggcgtacatcatcgccggagccatcgttgtgcttgttatgcaaatgctcggcgagatggctgctgcccgtcccgcctccggatcgttttcacgttacggcgaggatgctttcggccactgggctggtttctccctcggttggttgtactggttcatgctgattatggtgatgggcgccgaaatgactggcgctgctgccatcatgggtgcatggttcggcgtcgaaccgtggattccttcgcttgtctgcgtggtcttcttcgctgtggtgaacctcgtcgcggttcgcggtttcggtgaattcgagtactggttcgcattcattaaggtcgcggtgatcatcgctttcctcatcattggtattgctcttattttcggatggcttcccggatccacctttgtgggaacctcaaacttcatcggtgatcacggattcatgcccaatggtatttctggtgttgctgctggtttgctcgcggtggcttttgcctttggtggcattgaaattgtcaccattgcagctgcagagtccgataagccacgtgaagctatttccctggcggtgcgtgccgtgatttggcgtatttcagtcttttacttgggctctgttttggtcatcactttcctcatgccttatgagtcgatcaatggtgccgacaccgctgcggaatcccccttcacccaaatcctggcgatggcaaacatccctggcacggttggtttcatggaagcgatcatcgttctagcactgctttccgctttcaacgcccaaatctatgccacttctcgtttggtattttccatggcgaatcgacaagacgctccacgagttttcagtaagctcagcaccagccacgtccccaccaatgcggtgctgttgtccatgttcttcgccttcgtttcagttggtttgcagtactggaatccagccggtctgcttgatttcctcctcaacgctgttggcggttgtttgattgtggtgtgggcaatgatcactttgtcacagttgaaactccgcaaagaactgcaagcaaacggtgaaatctccacggttcgcatgtgggcgcacccatggttaggcatcctcaccttggttttgttggcaggactcgttgctctcatgctcggcgacgcagcctcccgcagccaggtttactcagtggcaattgtgtacggattcttggttcttttgtccttcgtcacagttaacagcccattgcgcggaggtcgcaccccttccgacttgaactga

SEQ ID NO: 3 - DNA, 490 bp, synthetic construct
  misc_feature 1..490: note = pyk promoter
  source 1..490: mol_type = other DNA
ctctacgtagctggttacaccttgggccgtttctggattgaacaaatgcgcgttgatgaagccacgcttattggcggcatccgaatcaacaccatcgtctccgcagtagtgtttgccggcgcgatcattgtgttcttcctgttgaagaagggtagggaaactcccgaagaggtagatccgactttcacagcgtctgttgcagcagatgctgtagcttcgccagatggaaaacccttgccgaaagcagaggagggcattgatggagaaacgccctcaacgcgataggtttcaaccataggcctgacctggctgagatgtttttggtagaaaaaccgagtgcccgaattgttttgtgggtgcccggtttttctgatttaagcacgtcagaggcgtagaacattgtctgttcacactctgggtcgcaagattcatcgagaattaatggtagtatctgtggcttgagggggaatgacgtactaggcttatgggc

SEQ ID NO: 4 - DNA, 502 bp, synthetic construct
  misc_feature 1..502: note = ald promoter
  source 1..502: mol_type = other DNA
cgatcatcgaactcggcgaagaaaaccgaaacctcaaagaatccctgcgtaaggtcacagctgagaatgagcagctcaaagatcaattacgcagcgggcgtccgcgtggcgagctggtgcacgtgccccgctccaccgcggtggtcatgtgggaacgccgcaaggggcgttccaagtaaaaacatgcttgtcgacgccactttctagcaaattaagcgggcacctccatttatcttttggaggtgcccgtttcgtgctttcgccaattagatacatggataaccacccgaacagggggtaataacttttgaaaggctttcggcgttgagctgcgagaattttgagaaaaagggggtgaatttaacaggggttctagcgcggattgattttcgtgaatatggtggctgctaagcgtgcgaatgtgcgcgttatcacaatcgttgaccaagtgtcacctgacgcacaggtagtgctcaggtggaggtggcccaaaggagaccca

SEQ ID NO: 5 - DNA, 45 bp, synthetic construct
  misc_feature 1..45: note = primer
  source 1..45: mol_type = other DNA
gctcggtacccggggatcctcattcgttcataattgatcccacag

SEQ ID NO: 6 - DNA, 19 bp, synthetic construct
  misc_feature 1..19: note = primer
  source 1..19: mol_type = other DNA
ggggagtgaatgctgggtg

SEQ ID NO: 7 - DNA, 24 bp, synthetic construct
  misc_feature 1..24: note = primer
  source 1..24: mol_type = other DNA
atggctaaatctaatgaagggctg

SEQ ID NO: 8 - DNA, 34 bp, synthetic construct
  misc_feature 1..34: note = primer
  source 1..34: mol_type = other DNA
tggagggtcggacgtccagaataatttctatcgg

SEQ ID NO: 9 - DNA, 27 bp, synthetic construct
  misc_feature 1..27: note = primer
  source 1..27: mol_type = other DNA
tctggacgtccgaccctccacgctgga

SEQ ID NO: 10 - DNA, 38 bp, synthetic construct
  misc_feature 1..38: note = primer
  source 1..38: mol_type = other DNA
cctgcaggtcgactctagagggctccttcgtcatcatc

SEQ ID NO: 11 - DNA, 38 bp, synthetic construct
  misc_feature 1..38: note = primer
  source 1..38: mol_type = other DNA
cccagcattcactccccctctacgtagctggttacacc

SEQ ID NO: 12 - DNA, 39 bp, synthetic construct
  misc_feature 1..39: note = primer
  source 1..39: mol_type = other DNA
ttcattagatttagccatgcccataagcctagtacgtca

SEQ ID NO: 13 - DNA, 37 bp, synthetic construct
  misc_feature 1..37: note = primer
  source 1..37: mol_type = other DNA
cccagcattcactcccccgatcatcgaactcggcgaa

SEQ ID NO: 14 - DNA, 36 bp, synthetic construct
  misc_feature 1..36: note = primer
  source 1..36: mol_type = other DNA
tcattagatttagccattgggtctcctttgggccac

SEQ ID NO: 15 - DNA, 23 bp, synthetic construct
  misc_feature 1..23: note = primer
  source 1..23: mol_type = other DNA
cgacatggaactaactctcctag

SEQ ID NO: 16 - DNA, 23 bp, synthetic construct
  misc_feature 1..23: note = primer
  source 1..23: mol_type = other DNA
cacttatgatcgctgtgatcagg

SEQ ID NO: 17 - DNA, 41 bp, synthetic construct
  misc_feature 1..41: note = primer
  source 1..41: mol_type = other DNA
cggggatcccccgggaggacggtactcaaatactaaacttc

SEQ ID NO: 18 - DNA, 38 bp, synthetic construct
  misc_feature 1..38: note = primer
  source 1..38: mol_type = other DNA
tgccgagtgtttcggtctttacagacacgagggacacg

SEQ ID NO: 19 - DNA, 31 bp, synthetic construct
  misc_feature 1..31: note = primer
  source 1..31: mol_type = other DNA
tgtctgtaaagaccgaaacactcggcatcaa

SEQ ID NO: 20 - DNA, 41 bp, synthetic construct
  misc_feature 1..41: note = primer
  source 1..41: mol_type = other DNA
cggggatcccccggggacaactacattattattataccaca

SEQ ID NO: 21 - DNA, 369 bp, synthetic construct
  misc_feature 1..369: note = ctaE promoter
  source 1..369: mol_type = other DNA
catgaatcgcattaagctgcaaaaacgccttttattcgggttcaaccaaaagttgtatgtggggctccaatggggtgaaaaactctgtgacgtgtctctcaggcaaaaacctgcggaaaccactttgggcacactctgtgagttcttcaaaatgggacgagtgtgatttgggacagattggaactgcctgtgaaccctttaacctgcaattatgtaactgtcgtaaaagggctatgaagagttcccggaaggtcgattgaaaagtttgcgaattgggggaaaattcgcatcaaaagccgagttcaaactttcaattgaaacggggggcttgaagtgactttggccaaccaaacagccatactagatagc

SEQ ID NO: 22 - DNA, 500 bp, synthetic construct
  misc_feature 1..500: note = pfkA promoter
  source 1..500: mol_type = other DNA
ttcttggcaagtgggtgggacaggccaaatgcaccaacgtaggttgccagcaggccagtagctactgcaggacccttcttttcattccagcttcgtgcagcaagcgctccggatgctgccaatggaatggtgcccagtgggcgaatgccggattcacgggcagtcaaccaaccgccgatcaaacctgctgcgacgacggtggcagtgctgacctgggatgcctttttcaatttcatttccatggtgagccagtctagagacaaaatttttccgcgggggttttcttgatctgatccgacaacccaatgggggcaaaaatgtgtccgaccaaaaattgtgcagcacaccacatgcccgctcggacaatgtcgatttgttaatgaaactgcagctctggcgattaaataagatggtcagagacagttttttggcctgtcaacccctgtgattctcttatttttgggtgattgttccggcgcgggtgttgtgatgggtttaat

SEQ ID NO: 23 - DNA, 5802 bp, synthetic construct
  misc_feature 1..5802: note = pDC24 vector
  source 1..5802: mol_type = other DNA
gttcgcttgctgtccataaaaccgcccagtctagctatcgccatgtaagcccactgcaagctacctgctttctctttgcgcttgcgttttcccttgtccagatagcccagtagctgacattcatccggggtcagcaccgtttctgcggactggctttctacgtgttccgcttcctttagcagcccttgcgccctgagtgcttgcggcagcgtgaagctagcttttatcgccattcgccattcaggctgcgcaactgttgggaagggcgatcggtgcgggcctcttcgctattacgccagctggcgaaagggggatgtgctgcaaggcgattaagttgggtaacgccagggttttcccagtcacgacgttgtaaaacgacggccagtgaattcgagctcggtacccggggatcctctagagtcgacctgcaggcatgcaagcttggcgtaatcatggtcatagctgtttcctgtgtgaaattgttatccgctcacaattccacacaacatacgagccggaagcataaagtgtaaagcctggggtgcctaatgagtgagctaactcacattaattgcgttgcgctcactgcccgctttccagtcgggaaacctgtcgtgccagctgcattaatgaatcggccaacgcgcggggagaggcggtttgcgtattgggcgctcttccgcttcctcgctcactgactcgctgcgctcggtcgttcggctgcggcgagcggtatcagctcactcaaaggcggtaatacggttatccacagaatcaggggataacgcaggaaagaacatgtgagcaaaaggccagcaaaaggccaggaaccgtaaaaaggccgcgttgctggcgtttttccataggctccgcccccctgacgagcatcacaaaaatcgacgctcaagtcagaggtggcgaaacccgacaggactataaagataccaggcgtttccccctggaagctccctcgtgcgctctcctgttccgaccctgccgcttaccggatacctgtccgcctttctcccttcgggaagcgtggcgctttctcaatgctcacgctgtaggtatctcagttcggtgtaggtcgttcgctccaagctgggctgtgtgcacgaaccccccgttcagcccgaccgctgcgccttatccggtaactatcgtcttgagtccaacccggtaagacacgacttatcgccactggcagcagccactggtaacaggattagcagagcgaggtatgtaggcggtgctacagagttcttgaagtggtggcctaactacggctacactagaaggacagtatttggtatctgcgctctgctgaagccagttaccttcggaaaaagagttggtagctcttgatccggcaaacaaaccaccgctggtagcggtggtttttttgtttgcaagcagcagattacgcgcagaaaaaaaggatctcaagaagatcctttgatcttttctacggggtctgacgctcagtggaacgaaaactcacgttaagggattttggtcatgagattatcaaaaaggatcttcacctagatccttttggggtgggcgaagaactccagcatgagatccccgcgctggaggatcatccagccctgatagaaacagaagccactggagcacctcaaaaacaccatcatacactaaatcagtaagttggcagcatcacccgacgcactttgcgccgaataaatacctgtgacggaagatcacttcgcagaataaataaatcctggtgtccctgttgataccgggaagccctgggccaacttttggcgaaaatgagacgttgatcggcacgtaagaggttccaactttcaccataatgaaataagatcactaccgggcgtattttttgagttatcgagattttcaggagctgatagaaacagaagccactggagcacctcaaaaacaccatcatacactaaatcagtaagttggcagcatcacccgacgcactttgcgccgaataaatacctgtgacggaagatcacttcgcagaataaataaatcctggtgtccctgttgataccgggaagccctgggccaacttttggcgaaaatgagacgttgatcggcacgtaagaggttccaactttcaccataatgaaataagatcactaccgggcgtattttttgagttatcgagattttcaggagctctttggcatcgtctctcgcctgtcccctcagttcagtaatttcctgcatttgcctgtttccagtcggtagatattccacaaaacagcagggaagcagcgcttttccgctgcataaccctgcttcggggtcattatagcgattttttcggtatatccatcctttttcgcacgatatacaggattttgccaaagggttcgtgtagactttccttggtgtatccaacggcgtcagccgggcaggataggtgaagtaggcccacccgcgagcgggtgttccttcttcactgtcccttattcgcacctggcggtgctcaacgggaatcctgctctgcgaggctggccggctaccgccggcgtaacagatgagggcaagcggatggctgatgaaaccaagccaaccaggaagggcagcccacctatcaaggtgtactgccttccagacgaacgaagagcgattgaggaaaaggcggcggcggccggcatgagcctgtcggcctacctgctggccgtcggccagggctacaaaatcacgggcgtcgtggactatgagcacgtccgcgagggcgtcccggaaaacgattccgaagcccaacctttcatagaaggcggcggtggaatcgaaatctcgtgatggcaggttgggcgtcgcttggtcggtcatttcgaaaaaggttaggaatacggttagccatttgcctgcttttatatagttcatatgggattcacctttatgttgataagaaataaaagaaaatgccaataggatatcggcattttcttttgcgtttttatttgttaactgttaattgtccttgttcaaggatgctgtctttgacaacagatgttttcttgcctttgatgttcagcaggaagctcggcgcaaacgttgattgtttgtctgcgtagaatcctctgtttgtcatatagcttgtaatcacgacattgtttcctttcgcttgaggtacagcgaagtgtgagtaagtaaaggttacatcgttaggcggatcaagatccatttttaacacaaggccagttttgttcagcggcttgtatgggccagttaaagaattagaaacataaccaagcatgtaaatatcgttagacgtaatgccgtcaatcgtcatttttgatccgcgggagtcagtgaacaggtaccatttgccgttcattttaaagacgttcgcgcgttcaatttcatctgttactgtgttagatgcaatcagcggtttcatcacttttttcagtgtgtaatcatcgtttagctcaatcataccgagagcgccgtttgctaactcagccgtgcgttttttatcgctttgcagaagtttttgactttcttgacggaagaatgatgtgcttttgccatagtatgctttgttaaataaagattcttcgccttggtagccatcttcagttccagtgtttgcttcaaatactaagtatttgtggcctttatcttctacgtagtgaggatctctcagcgtatggttgtcgcctgagctgtagttgccttcatcgatgaactgctgtacattttgatacgtttttccgtcaccgtcaaagattgatttataatcctctacaccgttgatgttcaaagagctgtctgatgctgatacgttaacttgtgcagttgtcagtgtttgtttgccgtaatgtttaccggagaaatcagtgtagaataaacggatttttccgtcagatgtaaatgtggctgaacctgaccattcttgtgtttggtcttttaggatagaatcatttgcatcgaatttgtcgctgtctttaaagacgcggccagcgtttttccagctgtcaatagaagtttcgccgactttttgatagaacatgtaaatcgatgtgtcatccgcatttttaggatctccggctaatgcaaagacgatgtggtagccgtgatagtttgcgacagtgccgtcagcgttttgtaatggccagctgtcccaaacgtccaggccttttgcagaagagatatttttaattgtggacgaatcaaattcagaaacttgatatttttcatttttttgctgttcagggatttgcagcatatcatggcgtgtaatatgggaaatgccgtatgtttccttatatggcttttggttcgtttctttcgcaaacgcttgagttgcgcctcctgccagcagtgcggtagtaaaggttaatactgttgcttgttttgcaaactttttgatgttcatcgttcatgtctccttttttatgtactgtgttagcggtctgcttcttccagccctcctgtttgaagatggcaagttagttacgcacaataaaaaaagacctaaaatatgtaaggggtgacgccaaagtatacactttgccctttacacattttaggtcttgcctgctttatcagtaacaaacccgcgcgatttacttttcgacctcattctattagactctcgtttggattgcaactggtctattttcctcttttgtttgatagaaaatcataaaaggatttgcagactacgggcctaaagaactaaaaaatctatctgtttcttttcattctctgtattttttatagtttctgttgcatgggcataaagttgcctttttaatcacaattcagaaaatatcataatatctcatttcactaaataatagtgaacggcaggtatatgtgatgggttaaaaaggatcaccccagagtcccgctcagaagaactcgtcaagaaggcgatagaaggcgatgcgctgcgaatcgggagcggcgataccgtaaagcacgaggaagcggtcagcccattcgccgccaagctcttcagcaatatcacgggtagccaacgctatgtcctgatagcggtccgccacacccagccggccacagtcgatgaatccagaaaagcggccattttccaccatgatattcggcaagcaggcatcgccatgggtcacgacgagatcctcgccgtcgggcatccgcgccttgagcctggcgaacagttcggctggcgcgagcccctgatgctcttcgtccagatcatcctgatcgacaagaccggcttccatccgagtacgtgctcgctcgatgcgatgtttcgcttggtggtcgaatgggcaggtagccggatcaagcgtatgcagccgccgcattgcatcagccatgatggatactttctcggcaggagcaaggtgagatgacaggagatcctgccccggcacttcgcccaatagcagccagtcccttcccgcttcagtgacaacgtcgagacagctgcgcaaggaacgcccgtcgtggccagccacgatagccgcgctgcctcgtcttggagttcattcagggcaccggacaggtcggtcttgacaaaaagaaccgggcgcccctgcgctgacagccggaacacggcggcatcagagcagccgattgtctgttgtgcccagtcatagccgaatagcctctccacccaagcggccggagaacctgcgtgcaatccatcttgttcaatcatgcgaaacgatcctcatcctgtctcttgatcagatcttgatcccctgcgccatcagatccttggcggcaagaaagccatccagtttactttgcagggcttcccaaccttaccagagggcgccccagctggcaattccg